European Patent Specification EP 3 556 860 B1, published March 6, 2024. Title: TYPE I-B CRISPR-CAS SYSTEM GENE CAS3-BASED GENE EDITING METHOD. Applicant: ANHUI UNIVERSITY. The sequence listing filed with the application follows.

SEQUENCE LISTING (54 sequences)

SEQ ID NO: 1 - DNA, 2316 bp, Streptomyces virginiae IBL14
gtgggccgtctggacgcggtggaggacgtcttcggcggcaggttctggcccgtcgtggaactcgctggcctcacccacgacgccggcaagattcccgaaggcttccagcggatgctggcgggatacagccgtgcctggggtgagcgtcacgaagtcgcctcgttgggcttcctgcccgcgctcatcggcgacccggacgtgctgttgtgggtggcgaccgcggtcgccacccaccatcgtccgctgaccggccagaacggacgcgacctgcagactctctacagcggtgtcaccatcaccgagctcgcgcaccgtttcgggccttttgacccacgcgctgtccccgccttggaggcctggcttcgtgcgagcgccatccgggtcggcctccccgcggccgctgttccagacgacggcacgctcaccgacaccggagtggtcgctggcgcccaccagctgctggaggagattttggaccgttgggcagaccgtgtgaggcctgaggtgggcttggccgctgtactgctgcagggggcggtcaccctggccgaccacttgtcctccgcccatcaggctctgcccaccgtccagccgttgggggccgggttccggtcccggttggagaaggagttcgctgaacgcggcaggaccctgcgtgcccaccagctggaggccgccaccgttaccggacatcttctgctgcgcgggccgaccggcagtgggaagaccgaggctgccctgctgtgggctgccagccaggtcgaggccctgaaggcggaaggccggggcgtgccgcgtgtgtttttcactctcccctacctggcctccatcaacgccatggcaacacggctgggtgacactctcggcgatggtgaggctgtcggcgttgcccactcccgcgccgcctcctaccaccttgcccaggccatcgccccgcaggacggcgacgaggaggacgaacacggagccccctgccgtgttgacgcggccgccaaggccttgtcccgggccgctgccaccaagctgttccgcgagagtgtccgcgtcgccaccccctaccagcttctgcgggccgccctggccgggccggcccactccggcatcctcatcgacgccgcgaactcggtgttcatcctggacgaactccacgcctacgacgcccgcaggctcggctacatcctggccagtgcccggctgtgggaacgcctcggtggacggatcacagtcctgtccgcgaccctgcccagggccctggccgacctgttcgagagcaccctcaccgcccccatcaccttcctcgacacccccgacctcgggctgccggcgcgccacctcctgcacacccgaggccaccatctcaccgacccggccacactggaggagatccgtctgcggctgtcccgggacgagtcggtcctggtgatcgccaacaacgtgtcccaggccatcgccctgtacgaacagctcgcacccgacgtgtgtgaacgcttcggtcaggacgccgcgctactgctgcactcccggtttcgacggatggaccggtcccggattgagcagaagatcgccgaccggttcgccactgtggcacctgatgcccagaacagccgtaagccgggcctggtcgttgccacgcaggtggtcgaggtcagtctcgacgtcgacttcgatgtgctgttcactggagcggctccgctcgaggccctcctgcagcgcttcggccggaccaaccgcgtcggggcccgcccgccggccgacgtcatcgtccaccatcccgcctggaccacacgccgccgacagcccggcgagtacgccgacggcatctacccacgggagccggtcgagtccgcgtggcacatcctcacccgcaatcacgggcgagtcatcgacgaagcggacgccaccgcgtggctggacgaggtctacgccacggactggggcaggcaatggcaccgcgaggtgctggagcggcgagaaagattcgaccgtgcgttcctgcagttccgctaccccttcgaagaccgcactgacctggccgataccttcgacgaactcttcgacggctccgaagccatcctcgccgaagaccaggacgcctactcagccgcactggccgcaccagacggcgaccaccccggagctggccggctcctcgcagaggaatacctcatccccgttccccactgggccagccccctcagccgctacgagaagcagctcaaagtccgcgtcatcaacggcgactaccaccccgaccacggcctcatggcggtccgggggctgccccagcccgcctaccgcgccggggaggtcttgtga

SEQ ID NO: 2 - protein, 771 aa, Streptomyces virginiae IBL14
VGRLDAVEDVFGGRFWPVVELAGLTHDAGKIPEGFQRMLAGYSRAWGERHEVASLGFLPALIGDPDVLLWVATAVATHHRPLTGQNGRDLQTLYSGVTITELAHRFGPFDPRAVPALEAWLRASAIRVGLPAAAVPDDGTLTDTGVVAGAHQLLEEILDRWADRVRPEVGLAAVLLQGAVTLADHLSSAHQALPTVQPLGAGFRSRLEKEFAERGRTLRAHQLEAATVTGHLLLRGPTGSGKTEAALLWAASQVEALKAEGRGVPRVFFTLPYLASINAMATRLGDTLGDGEAVGVAHSRAASYHLAQAIAPQDGDEEDEHGAPCRVDAAAKALSRAAATKLFRESVRVATPYQLLRAALAGPAHSGILIDAANSVFILDELHAYDARRLGYILASARLWERLGGRITVLSATLPRALADLFESTLTAPITFLDTPDLGLPARHLLHTRGHHLTDPATLEEIRLRLSRDESVLVIANNVSQAIALYEQLAPDVCERFGQDAALLLHSRFRRMDRSRIEQKIADRFATVAPDAQNSRKPGLVVATQVVEVSLDVDFDVLFTGAAPLEALLQRFGRTNRVGARPPADVIVHHPAWTTRRRQPGEYADGIYPREPVESAWHILTRNHGRVIDEADATAWLDEVYATDWGRQWHREVLERRERFDRAFLQFRYPFEDRTDLADTFDELFDGSEAILAEDQDAYSAALAAPDGDHPGAGRLLAEEYLIPVPHWASPLSRYEKQLKVRVINGDYHPDHGLMAVRGLPQPAYRAGEVL

SEQ ID NO: 3 - DNA, 1144 bp, Artificial Sequence
  The sequence is synthetized.
atgagcgtggtggttatgccgatcgcgtcacactacgtctgaacgtcgaaaacccgaaactgtggagcgccgaaatcccgaatctctatcgtgcggtggttgaactgcacaccgccgacggcacgctgattgaagcagaagcctgcgatgtcggtttccgcgaggtgcggattgaaaatggtctgctgctgctgaacggcaagccgttgctgattcgaggcgttaaccgtcacgagcatcatcctctgcatggtcaggtcatggatgagcagacgatggtgcaggatatcctgctgatgaagcagaacaactttaacgccgtgcgctgttcgcattatccgaaccatccgctgtggtacacgctgtgcgaccgctacggcctgtatgtggtggatgaagccaatattgaaacccacggcatgggtttacagggcggcttcgtctgggactgggtggatcagtcgctgattaaatatgatgaaaacggcaacccgtggtcggcttacggcggtgattttggcgatacgccgaacgatcgccagttctgtatgaacggtctggtctttgccgaccgcacgccgcatccagcgctgacggaagcaaaacaccagcagcagtttttccagttccgtttatccgggcaaaccatcgaagtgaccagcgaatacctgttccgtcatagcgataacgagctcctgcactggatggtggcgctggatggtaagccgctggcaagcggtgaagtgcctctggatgtcgctccacaaggtaaacagttgattgaactgcctgaactaccgcagccggagagcgccgggcaactctggctcacagtacgcgtagtgcaaccgaacgcgaccgcatggtcagaagccgggcacatcagcgcctggcagcagtggcgtctggcggaaaacctcagtgtgacgctccccgccgcgtcccacgccatcccgcatctgaccaccagcgaaatggatttttgcatcgagctgggtaataagcgttggcaatttaaccgccagtcaggctttctttcacagatgtggattggcgataaaaaacaactgctgacgccgctgcgcgatcagttcacccgtgcaccgctggataacgacattggcgtaagtgaagcgacccgcat

SEQ ID NO: 4 - DNA, 222 bp, Artificial Sequence
  The sequence is synthetized.
ggctgcaggtcgactctagaggatcctaatacgactcactatagggaatattgtcctcatcgccccttcgaggggtcgcaacccgcccggtgcagtatgaaggcggcggagccgacaccacggtcctcatcgccccttcgaggggtcgcaacataaaacgaaaggctcagtcgaaagactgggcctttcgttttatgaattcgtaatcatgtcatagctgtt

SEQ ID NO: 5 - DNA, 46 bp, Artificial Sequence
  The sequence is synthetized.
actttttattttaggaggcaaaagtgggccgtctggacgcggtgga

SEQ ID NO: 6 - DNA, 50 bp, Artificial Sequence
  The sequence is synthetized.
aaataatcttcatctaaaatatactttcacaagacctccccggcgcggta

SEQ ID NO: 7 - DNA, 27 bp, Artificial Sequence
  The sequence is synthetized.
tacccaacttaatcgccttgcagcaca

SEQ ID NO: 8 - DNA, 28 bp, Artificial Sequence
  The sequence is synthetized.
ccgtcgatattcagccatgtgccttctt

SEQ ID NO: 9 - DNA, 50 bp, Artificial Sequence
  The sequence is synthetized.
taccgcgccggggaggtcttgtgaaagtatattttagatgaagattattt

SEQ ID NO: 10 - DNA, 46 bp, Artificial Sequence
  The sequence is synthetized.
tccaccgcgtccagacggcccacttttgcctcctaaaataaaaagt

SEQ ID NO: 11 - DNA, 46 bp, Artificial Sequence
  The sequence is synthetized.
gtaaaacgacggccagtgccaagcttatgagcgtggtggttatgcc

SEQ ID NO: 12 - DNA, 39 bp, Artificial Sequence
  The sequence is synthetized.
acgaagccgccctgtaaacccatgccgtgggtttcaata

SEQ ID NO: 13 - DNA, 39 bp, Artificial Sequence
  The sequence is synthetized.
tattgaaacccacggcatgggtttacagggcggcttcgt

SEQ ID NO: 14 - DNA, 46 bp, Artificial Sequence
  The sequence is synthetized.
tcgcgcgcggccgcggatcctctagaatgcgggtcgcttcacttac

SEQ ID NO: 15 - DNA, 1397 bp, Artificial Sequence
  The sequence is synthetized.
gtgatggatttaaaccacggaaaggcgtttgcgccacaaccggtcaaaacatcttacggaacatatgaagactgcaaggatgctgatattgtctgcatttgcgccggagcaaaccaaaaacctggtgagacacgccttgaattagtagaaaagaacttgaagattttcaaaggcatcgttagtgaagtcatggcgagcggatttgacggcattttcttagtcgcgacaaatccggttgatatcctgacttacgcaacatggcgcgcctacctgtgacggaagatcacttcgcagaataaataaatcctggtgtccctgttgataccgggaagccctgggccaacttttggcgaaaatgagacgttgatcggcacgtaagaggttccaactttcaccataatgaaataagatcactaccgggcgtattttttgagttgtcgagattttcaggagctaaggaagctaaaatggagaaaaaaatcactggatataccaccgttgatatatcccaatggcatcgtaaagaacattttgaggcatttcagtcagttgctcaatgtacctataaccagaccgttcagctggatattacggcctttttaaagaccgtaaagaaaaataagcacaagttttatccggcctttattcacattcttgcccgcctgatgaatgctcatccggaattccgtatggcaatgaaagacggtgagctggtgatatgggatagtgttcacccttgttacaccgttttccatgagcaaactgaaacgttttcatcgctctggagtgaataccacgacgatttccggcagtttctacacatatattcgcaagatgtggcgtgttacggtgaaaacctggcctatttccctaaagggtttattgagaatatgtttttcgtctcagccaatccctgggtgagtttcaccagttttgatttaaacgtggccaatatggacaacttcttcgcccccgttttcaccatgggcaaatattatacgcaaggcgacaaggtgctgatgccgctggcgattcaggttcatcatgccgtctgtgatggcttccatgtcggcagaatgcttaatgaattacaacagtactgcgatgagtggcagggcggggcgtaaggcgcgccatttaaatgaagttcctattccgaagttcccgatgcgtacaaacaagaggagctggaccaaattgtagatgatgtgaaaaacgcagcttaccatatcattgagaaaaaaggcgcgacttattatggggttgcgatgagtcttgctcgcattacaaaagccattcttcataatgaaaacagcatattaactgtcagcacatatttggacgggcaatacggtgcagatgacgtgtacatcggtgtgccggctgtcgtgaatcgc

SEQ ID NO: 16 - DNA, 291 bp, Artificial Sequence
  The sequence is synthetized.
ggctgcaggtcgactctagaggatcctaatgtgagttagctcactcattaggcaccccaggctttacactttatgcttccggctcgtatgttgtgtggaattgtgagcggataacaagtcctcatcgccccttcgaggggtcgcaacagcggcctgccaaaagagcgggtgattggaagcggcacaagtcctcatcgccccttcgaggggtcgcaacctagcataaccccttggggcctctaaacgggtcttgaggggttttttggaattcgtaatcatgtcatagctgtt

SEQ ID NO: 17 - DNA, 19 bp, Artificial Sequence
  The sequence is synthetized.
atgatgaacaaacatgtaa

SEQ ID NO: 18 - DNA, 18 bp, Artificial Sequence
  The sequence is synthetized.
ttagttgactttttgttc

SEQ ID NO: 19 - DNA, 46 bp, Artificial Sequence
  The sequence is synthetized.
taacaatttcacacaggaaacagctgtggtcgccggtgccccgaac

SEQ ID NO: 20 - DNA, 45 bp, Artificial Sequence
  The sequence is synthetized.
ttggcgggtgtcggggctggcttaatcacaagacctccccggcgc

SEQ ID NO: 21 - DNA, 47 bp, Artificial Sequence
  The sequence is synthetized.
gtaaaacgacggccagtgccaagcttcgatgagatggatttaaacca

SEQ ID NO: 22 - DNA, 40 bp, Artificial Sequence
  The sequence is synthetized.
tttttctcaacgagttcactatgttgcgtaagtcaggata

SEQ ID NO: 23 - DNA, 36 bp, Artificial Sequence
  The sequence is synthetized.
tatcctgacttacgcaacatggcgcgcctacctgtg

SEQ ID NO: 24 - DNA, 36 bp, Artificial Sequence
  The sequence is synthetized.
cacaggtaggcgcgccatgttgcgtaagtcaggata

SEQ ID NO: 25 - DNA, 40 bp, Artificial Sequence
  The sequence is synthetized.
tatcctgacttacgcaacatagtgaactcgttgagaaaaa

SEQ ID NO: 26 - DNA, 42 bp, Artificial Sequence
  The sequence is synthetized.
tcgcgcgcggccgcggatcctctagagcgattcacgacagcc

SEQ ID NO: 27 - DNA, 807 bp, Artificial Sequence
  The sequence is synthetized.
cagccattccattggagtttactccacaagatgatattgttttgttggaaccatatcattatttgggaaaaaatcctggtaaagaaattcgttcacaattgattgaagcctttaattattggttggatgttaaaaaagaggaccttgaagttattcaaaatgttgttggtatgttgcatactgcttctttgctcatggatgatgttgaagatagttccgttttacgtcggggttcaccagttgctcatttgatctacggtattccacaaactattaatacagccaattatgtttactttttagcctatcaagaaatttttaaattgcgtccaacacctattcctatgccagttggtggtttgtttcgtattgccgttcgtttgatgatggccaaatctgaatgtgatattgattttgttcaattagttaatttgattagtatctattttcaaattcgtgatgattatatgaatcttcaatctagtgaatatgcacataacaaaaattttgccgaggaccttactgaaggtaaattttcctttccaactattcatagtattcatactaatccaagtagtcgtttagttattaatacattacagaaaaaatctacatccccagaaattttgcatcattgtgttaattatatgcgtactgaaacacattcctttgaatatactcgtgaagttttgaatactttgtccggtgccttggaacgtgaattgggtcgtttgcaagaagaatttgccgaagctaatagtcgtatggatttgggcgacgttgaatccgaaggtcgtacagggaaaa

SEQ ID NO: 28 - DNA, 406 bp, Artificial Sequence
  The sequence is synthetized.
cggaattctctttgaaaagataatgtatgattatgctttcactcatatttatacagaaacttgatgttttctttcgagtatatacaaggtgattacatgtacgtttgaagtacaactctagattttgtagtgccctcttgggctagcggtaaaggtgcgcattttttcacaccctacaatgttctgttcaaaagattttggtcaaacgctgtagaagtgaaagttggtgcgcatgtttcggcgttcgaaacttctccgcagtgaaagataaatgatcgtcctcatcgccccttcgaggggtcgcaactagtgcctcatcttcttcttcagcatcctccgaaaatggtgtcctcatcgccccttcgaggggtcgcaactttttttgttttttatgtctctcgagcgg

SEQ ID NO: 29 - DNA, 23 bp, Artificial Sequence
  The sequence is synthetized.
cagcatacacctcactagggtag

SEQ ID NO: 30 - DNA, 22 bp, Artificial Sequence
  The sequence is synthetized.
ccccttccagtgcattatgcaa

SEQ ID NO: 31 - DNA, 34 bp, Artificial Sequence
  The sequence is synthetized.
cccaagcttcagccattccattggagtttactcc

SEQ ID NO: 32 - DNA, 50 bp, Artificial Sequence
  The sequence is synthetized.
aacggcaatacgaaacaaaccaccaactggcataggaataggtgttggac

SEQ ID NO: 33 - DNA, 50 bp, Artificial Sequence
  The sequence is synthetized.
gtccaacacctattcctatgccagttggtggtttgtttcgtattgccgtt

SEQ ID NO: 34 - DNA, 33 bp, Artificial Sequence
  The sequence is synthetized.
cgcggatccttttccctgtacgaccttcggatt

SEQ ID NO: 35 - DNA, 39 bp, Artificial Sequence
  The sequence is synthetized.
tatagggccggtgaagttttaagcagggctgaccccaag

SEQ ID NO: 36 - DNA, 48 bp, Artificial Sequence
  The sequence is synthetized.
caacggcatccaatctacccatttttttcccgggggatccactagttc

SEQ ID NO: 37 - DNA, 28 bp, Artificial Sequence
  The sequence is synthetized.
aaaaaaatgggtagattggatgccgttg

SEQ ID NO: 38 - DNA, 38 bp, Artificial Sequence
  The sequence is synthetized.
gtcagccctgcttaaaacttcaccggccctatatgcag

SEQ ID NO: 39 - DNA, 1972 bp, Artificial Sequence
  The sequence is synthetized.
tggcttgactagggggtctttgagttgctcatcaagatggtcaggcatttatgaaaccctgtttacatagtaagaattattttttaaaaaaacttttccctttttcttttctgccatgaagtcacagaatgtcgttccacccgggacgagggtgtccccgaggacgaggaggacatggagccagaccctcagcaccatcctttaggccccaaaatctgaggctgcttcaccctcagcagcctcctgtgcaatatcaatatgaacctccaataagatacattgatgagtttggacaaaccacaactagaatgcagtgaaaaaaatgctttatttgtgaaatttgtgatgctattgctttatttgtaaccattataagctgcaataaacaagttggggtgggcgaagaactccagcatgagatccccgcgctggaggatcatccagccggcgtcccggaaaacgattccgaagcccaacctttcatagaaggcggcggtggaatcgaaatctcgtagcacgtgctattcctttgccctcggacgagtgctggggcgtcggtttccactatcggcgagtacttctacacagccatcggtccagacggccgcgcttctgcgggcgatttgtgtacgcccgacagtcccggctccggatcggacgattgcgtcgcatcgaccctgcgcccaagctgcatcatcgaaattgccgtcaaccaagctctgatagagttggtcaagaccaatgcggagcatatacgcccggagccgcggcgatcctgcaagctccggatgcctccgctcgaagtagcgcgtctgctgctccatacaagccaaccacggcctccagaagaagatgttggcgacctcgtattgggaatccccgaacatcgcctcgctccagtcaatgaccgctgttatgcggccattgtccgtcaggacattgttggagccgaaatccgcgtgcacgaggtgccggacttcggggcagtcctcggcccaaagcatcagctcatcgagagcctgcgcgacggacgcactgacggtgtcgtccatcacagtttgccagtgatacacatggggatcagcaatcgcgcatatgaaatcacgccatgtagtgtattgaccgattccttgcggtccgaatgggccgaacccgctcgtctggctaagatcggccgcagcgatcgcatccatggcctccgcgaccggctgcagaacagcgggcagttcggtttcaggcaggtcttgcaacgtgacaccctgtgcacggcgggagatgcaataggtcaggctctcgctgaattccccaatgtcaagcacttccggaatcgggagcgcggccgatgcaaagtgccgataaacataacgatctttgtagaaaccatcggcgcagctatttacccgcaggacatatccacgccctcctacatcgaagctgaaagcacgagattcttcgccctccgagagctgcatcaggtcggagacgctgtcgaacttttcgatcagaaacttctcgacagacgtcgcggtgagttcaggctttttcatcacgtgctgatcagatccgaaaatggatatacaagctcccgggagctttttgcaaaagcctaggcctccaaaaaagcctccccactacttctggaatagctcagaggcagaggcggcctcggcctctgcataaataaaaaaaattagtcagccatggggcggagaatgggcggaactgggcggagttaggggcgggatgggcggagttaggggcgggactatggttgctgactaattgagatgcacagactttgtacccttccccccacccatgcctccgtcagcgcaaggccctcttcccccctgcccaatcaggccgcctttccccaaccaccagatgaggcaccccttcccagttcctccttgttttcctcccatgccaccaccaatgccttgtcctaataaccccccagtccctggggcac

SEQ ID NO: 40 - DNA, 166 bp, Artificial Sequence
  The sequence is synthetized.
taatacgactcactatagggaatattgtcctcatcgccccttcgaggggtcgcaaccaccactttctcaaactctccagcccccaattttctgtcctcatcgccccttcgaggggtcgcaacataaaacgaaaggctcagtcgaaagactgggcctttcgttttat

SEQ ID NO: 41 - DNA, 16 bp, Artificial Sequence
  The sequence is synthetized.
accgcgcacaaggccc

SEQ ID NO: 42 - DNA, 39 bp, Artificial Sequence
  The sequence is synthetized.
taagacagatgactgacattccacctaattaatatccca

SEQ ID NO: 43 - DNA, 24 bp, Artificial Sequence
  The sequence is synthetized.
tgcactccagcttagggacagagt

SEQ ID NO: 44 - DNA, 45 bp, Artificial Sequence
  The sequence is synthetized.
caattaccataacactaattttgtagtttccaatacacttagcct

SEQ ID NO: 45 - DNA, 25 bp, Artificial Sequence
  The sequence is synthetized.
tggagcagctttaaggaatggtcgg

SEQ ID NO: 46 - DNA, 17 bp, Artificial Sequence
  The sequence is synthetized.
ctcgctcccgccgatcc

SEQ ID NO: 47 - DNA, 36 bp, Artificial Sequence
  The sequence is synthetized.
acacaggaaacagcttgcactccagcttagggacag

SEQ ID NO: 48 - DNA, 46 bp, Artificial Sequence
  The sequence is synthetized.
tttttcatcaattaccataacactaattttgtagtttccaatacac

SEQ ID NO: 49 - DNA, 30 bp, Artificial Sequence
  The sequence is synthetized.
gtaattgatgaaaaagcctgaactcaccgc

SEQ ID NO: 50 - DNA, 29 bp, Artificial Sequence
  The sequence is synthetized.
ctgctccactattcctttgccctcggacg

SEQ ID NO: 51 - DNA, 31 bp, Artificial Sequence
  The sequence is synthetized.
ggaatagtggagcagctttaaggaatggtcg

SEQ ID NO: 52 - DNA, 30 bp, Artificial Sequence
  The sequence is synthetized.
tcggggctggcttaactcgctcccgccgat

SEQ ID NO: 53 - DNA, 30 bp, Artificial Sequence
  The sequence is synthetized.
gccgccgcgatcgccgtgggccgtctggac

SEQ ID NO: 54 - DNA, 32 bp, Artificial Sequence
  The sequence is synthetized.
gcgttttttcttgggtcacaagacctccccgg